European Patent Application EP 4 299 751 A1, published January 3, 2024. Title: Method of production of recombinant AAV9 virion. Applicant: JCR Pharmaceuticals Co., Ltd. The sequence listing filed with the application follows.

SEQUENCE LISTING (10 sequences)

SEQ ID NO: 1 - DNA, 2168 bp, Artificial Sequence
  Nucleic acid sequence containing the SalI site, RsrII site, ColE1 ori, ampicillin resistance gene, BsiWI site, BstZ17I site, and BsrGI site, synthetic sequence
gtcgacgtttaaaccatatgatcagctcactcaaaggcggtaatacgcggaccggctatggctcggaccggttatccacagaatcaggggataacgcaggaaagaacatgtgagcaaaaggccagcaaaaggccaggaaccgtaaaaaggccgcgttgctggcgtttttccataggctccgcccccctgacgagcatcacaaaaatcgacgctcaagtcagaggtggcgaaacccgacaggactataaagataccaggcgtttccccctggaagctccctcgtgcgctctcctgttccgaccctgccgcttaccggatacctgtccgcctttctcccttcgggaagcgtggcgctttctcatagctcacgctgtaggtatctcagttcggtgtaggtcgttcgctccaagctgggctgtgtgcacgaaccccccgttcagcccgaccgctgcgccttatccggtaactatcgtcttgagtccaacccggtaagacacgacttatcgccactggcagcagccactggtaacaggattagcagagcgaggtatgtaggcggtgctacagagttcttgaagtggtggcctaactacggctacactagaagaacagtatttggtatctgcgctctgctgaagccagttaccttcggaaaaagagttggtagctcttgatccggcaaacaaaccaccgctggtagcggtggtttttttgtttgcaagcagcagattacgcgcagaaaaaaaggatctcaagaagatcctttgatcttttctacggggtctgacgctcagtggaacgaaaactcacgttaagggattttggtcatgagattatcaaaaaggatcttcacctagatccttttaaattaaaaatgaagttttaaatcaatctaaagtatatatgagtaaacttggtctgacagttaccaatgcttaatcagtgaggcacctatctcagcgatctgtctatttcgttcatccatagttgcctgactccccgtcgtgtagataactacgatacgggagggcttaccatctggccccagtgctgcaatgataccgcgagacccacgctcaccggctccagatttatcagcaataaaccagccagccggaagggccgagcgcagaagtggtcctgcaactttatccgcctccatccagtctattaattgttgccgggaagctagagtaagtagttcgccagttaatagtttgcgcaacgttgttgccattgctacaggcatcgtggtgtcacgctcgtcgtttggtatggcttcattcagctccggttcccaacgatcaaggcgagttacatgatcccccatgttgtgcaaaaaagcggttagctccttcggtcctccgatcgttgtcagaagtaagttggccgcagtgttatcactcatggttatggcagcactgcataattctcttactgtcatgccatccgtaagatgcttttctgtgactggtgagtactcaaccaagtcattctgagaatagtgtatgcggcgaccgagttgctcttgcccggcgtcaatacgggataataccgcgccacatagcagaactttaaaagtgctcatcattggaaaacgttcttcggggcgaaaactctcaaggatcttaccgctgttgagatccagttcgatgtaacccactcgtgcacccaactgatcttcagcatcttttactttcaccagcgtttctgggtgagcaaaaacaggaaggcaaaatgccgcaaaaaagggaataagggcgacacggaaatgttgaatactcatactcttcctttttcaatattattgaagcatttatcagggttattgtctcatgagcggatacatatttgaatgtatttagaaaaataaacaaataggggttccgcgcacatttccccgaaaagtgccacctcgtacggcctgagtgtatacccgttacggacatggatccggtacccaactccatgcttaacagtccccaggtacagcccaccctgcgtcgcaaccaggaacagctctacagcttcctggagcgccactcgccctacttccgcagccacagtgcgcagattaggagcgccacttctttttgtcacttgaaaaacatgtaaaaataatgtactaggagacactttcaataaaggcaaatgtttttatttgtaca

SEQ ID NO: 2 - DNA, 2559 bp, Artificial Sequence
  Nucleic acid sequence containing the ClaI site, human CMV enhancer, chicken beta actin promoter, chicken beta actin/MVM chimeric intron, palmitoyl-protein thioesterase 1(PPT1) gene, WPRE, bGH poly A sequence, and BglII site, synthetic sequence
atcgatatcaagctttagttattaatagtaatcaattacggggtcattagttcatagcccatatatggagttccgcgttacataacttacggtaaatggcccgcctggctgaccgcccaacgacccccgcccattgacgtcaataatgacgtatgttcccatagtaacgccaatagggactttccattgacgtcaatgggtggagtatttacggtaaactgcccacttggcagtacatcaagtgtatcatatgccaagtacgccccctattgacgtcaatgacggtaaatggcccgcctggcattatgcccagtacatgaccttatgggactttcctacttggcagtacatctacgtattagtcatcgctattaccatggtcgaggtgagccccacgttctgcttcactctccccatctcccccccctccccacccccaattttgtatttatttattttttaattattttgtgcagcgatgggggcggggggggggggggggcgcgcgccaggcggggcggggcggggcgaggggcggggcggggcgaggcggagaggtgcggcggcagccaatcagagcggcgcgctccgaaagtttccttttatggcgaggcggcggcggcggcggccctataaaaagcgaagcgcgcggcgggcggggagtcgctgcgttgccttcgccccgtgccccgctccgcgccgcctcgcgccgcccgccccggctctgactgaccgcgttactcccacaggtgagcgggcgggacggcccttctcctccgggctgtaattagcaagaggtaagggtttaagggatggttggttggtggggtattaatgtttaattacctggagcacctgcctgaaatcactttttttcaggttggttaattaaacgcgtggtacctctagagtcgaggccaccatggcgtcgcccggctgcctgtggctcttggctgtggctctcctgccatggacctgcgcttctcgggcgctgcagcatctggacccgccggcgccgctgccgttggtgatctggcatgggatgggagacagctgttgcaatcccttaagcatgggtgctattaaaaaaatggtggagaagaaaatacctggaatttacgtcttatctttagagattgggaagaccctgatggaggacgtggagaacagcttcttcttgaatgtcaattcccaagtaacaacagtgtgtcaggcacttgctaaggatcctaaattgcagcaaggctacaatgctatgggattctcccagggaggccaatttctgagggcagtggctcagagatgcccttcacctcccatgatcaatctgatctcggttgggggacaacatcaaggtgtttttggactccctcgatgcccaggagagagctctcacatctgtgacttcatccgaaaaacactgaatgctggggcgtactccaaagttgttcaggaacgcctcgtgcaagccgaatactggcatgaccccataaaggaggatgtgtatcgcaaccacagcatcttcttggcagatataaatcaggagcggggtatcaatgagtcctacaagaaaaacctgatggccctgaagaagtttgtgatggtgaaattcctcaatgattccattgtggaccctgtagattcggagtggtttggattttacagaagtggccaagccaaggaaaccattcccttacaggagacctccctgtacacacaggaccgcctggggctaaaggaaatggacaatgcaggacagctagtgtttctggctacagaaggggaccatcttcagttgtctgaagaatggttttatgcccacatcataccattccttggataagcggccgcgcgatcgccgggtggcatccctgtgacccctccccagtgcctctcctggccctggaagttgccactccagtgcccaccagccttgtcctaataaaattaagttgcatcattttgtctgactaggtgtccttctataatattatggggtggaggggggtggtatggagcaaggggcaagttgggaagacaacctgtagggcctgcggggtctattgggaaccaagctggagtgcagtggcacaatcttggctcactgcaatctccgcctcctgggttcaagcgattctcctgcctcagcctcccgagttgttgggattccaggcatgcatgaccaggctcagctaatttttgtttttttggtagagacggggtttcaccatattggccaggctggtctccaactcctaatctcaggtgatctacccaccttggcctcccaaattgctgggattacaggcgtgaaccactgctcccttccctgtccttatttaaatctgtgccttctagttgccagccatctgttgtttgcccctcccccgtgccttccttgaccctggaaggtgccactcccactgtcctttcctaataaaatgaggaaattgcatcgcattgtctgagtaggtgtcattctattctggggggtggggtggggcaggacagcaagggggaggattgggaagacaatagcaggcatgctggggaagatct

SEQ ID NO: 3 - DNA, 2820 bp, Artificial Sequence
  Nucleic acid sequence containing AfeI site, RsrII site, BsrGI site, AvrII site, ampicillin resistance gene, ColE1 ori, RsrII site, 5' part of Rep region of serotype 2 AAV (including p5 promoter), and SacII site, synthetic sequence
agcgctcggaccgggcgcgctcactggccgtcgttttacaacgtcgtgactgggaaaaccctgtacaggctgaccggtgttgcctaggtgaatggcgaatggtcaggtggcacttttcggggaaatgtgcgcggaacccctatttgtttatttttctaaatacattcaaatatgtatccgctcatgagacaataaccctgataaatgcttcaataatattgaaaaaggaagagtatgagtattcaacatttccgtgtcgcccttattcccttttttgcggcattttgccttcctgtttttgctcacccagaaacgctggtgaaagtaaaagatgctgaagatcagttgggtgcacgagtgggttacatcgaactggatctcaacagcggtaagatccttgagagttttcgccccgaagaacgttttccaatgatgagcacttttaaagttctgctatgtggcgcggtattatcccgtattgacgccgggcaagagcaactcggtcgccgcatacactattctcagaatgacttggttgagtactcaccagtcacagaaaagcatcttacggatggcatgacagtaagagaattatgcagtgctgccataaccatgagtgataacactgcggccaacttacttctgacaacgatcggaggaccgaaggagctaaccgcttttttgcacaacatgggggatcatgtaactcgccttgatcgttgggaaccggagctgaatgaagccataccaaacgacgagcgtgacaccacgatgcctgtagcaatggcaacaacgttgcgcaaactattaactggcgaactacttactctagcttcccggcaacaattaatagactggatggaggcggataaagttgcaggaccacttctgcgctcggcccttccggctggctggtttattgctgataaatctggagccggtgagcgtgggtctcgcggtatcattgcagcactggggccagatggtaagccctcccgtatcgtagttatctacacgacggggagtcaggcaactatggatgaacgaaatagacagatcgctgagataggtgcctcactgattaagcattggtaactgtcagaccaagtttactcatatatactttagattgatttaaaacttcatttttaatttaaaaggatctaggtgaagatcctttttgataatctcatgaccaaaatcccttaacgtgagttttcgttccactgagcgtcagaccccgtagaaaagatcaaaggatcttcttgagatcctttttttctgcgcgtaatctgctgcttgcaaacaaaaaaaccaccgctaccagcggtggtttgtttgccggatcaagagctaccaactctttttccgaaggtaactggcttcagcagagcgcagataccaaatactgttcttctagtgtagccgtagttaggccaccacttcaagaactctgtagcaccgcctacatacctcgctctgctaatcctgttaccagtggctgctgccagtggcgataagtcgtgtcttaccgggttggactcaagacgatagttaccggataaggcgcagcggtcgggctgaacggggggttcgtgcacacagcccagcttggagcgaacgacctacaccgaactgagatacctacagcgtgagctatgagaaagcgccacgcttcccgaagggagaaaggcggacaggtatccggtaagcggcagggtcggaacaggagagcgcacgagggagcttccagggggaaacgcctggtatctttatagtcctgtcgggtttcgccacctctgacttgagcgtcgatttttgtgatgctcgtcaggggggcggagcctatggaaaaacgccagcaacgcggcctttttacggttcctggccttttgctggccttttgctcacatgttctttcctgcgttatcccctgattctgtggataaccgtattaccgcctttgagtgagctgataccgctcgccgcagccgaacgaccgagcgcagcgagtcagtgagcgaggaagcggaagagcgcccaatacgcaaaccgcctctccccgcgcgttggccgattcattaatgcagctggcacgacaggtttcccgactggaaagcgggcagtgagcgcaacgcaattaatgtgagttagctcactcattaggcaccccaggctttacactttatgcttccggctcgtatgttgtgtggaattgtgagcggataacaatttcacacaggaaacagctatgaccatgattacgccaacggaccgggaggggtggagtcgtgacgtgaattacgtcatagggttagggaggtcctgtattagaggtcacgtgagtgttttgcgacattttgcgacaccatgtggtctcgctgggggggggggcccgagtgagcacgcagggtctccattttgaagcgggaggtttgaacgcgcagccgccacgccggggttttacgagattgtgattaaggtccccagcgaccttgacgagcatctgcccggcatttctgacagctttgtgaactgggtggccgagaaggaatgggagttgccgccagattctgacatggatctgaatctgattgagcaggcacccctgaccgtggccgagaagctgcagcgcgactttctgacggaatggcgccgtgtgagtaaggccccggaggcccttttctttgtgcaatttgagaagggagagagctacttccacatgcacgtgctcgtggaaaccaccggggtgaaatccatggttttgggacgtttcctgagtcagattcgcgaaaaactgattcagagaatttaccgcgg

SEQ ID NO: 4 - DNA, 2911 bp, Artificial Sequence
  Nucleic acid sequence containing HindIII site, 3' part of Rep region of serotype 2 AAV, Cap region of serotype 9 AAV, p5 promoter, RsrII site, and BsrGI site, synthetic sequence
aagcttcgatcaactacgcagacaggtaccaaaacaaatgttctcgtcacgtgggcatgaatctgatgctgtttccctgcagacaatgcgagagaatgaatcagaattcaaatatctgcttcactcacggacagaaagactgtttagagtgctttcccgtgtcagaatctcaacccgtttctgtcgtcaaaaaggcgtatcagaaactgtgctacattcatcatatcatgggaaaggtgccagacgcttgcactgcctgcgatctggtcaatgtggatttggatgactgcatctttgaacaataaatgatttaaatcaggtatggctgccgatggttatcttccagattggctcgaggacaaccttagtgaaggaattcgcgagtggtgggctttgaaacctggagcccctcaacccaaggcaaatcaacaacatcaagacaacgctcgaggtcttgtgcttccgggttacaaataccttggacccggcaacggactcgacaagggggagccggtcaacgcagcagacgcggcggccctcgagcacgacaaggcctacgaccagcagctcaaggccggagacaacccgtacctcaagtacaaccacgccgacgccgagttccaggagcggctcaaagaagatacgtcttttgggggcaacctcgggcgagcagtcttccaggccaaaaagaggcttcttgaacctcttggtctggttgaggaagcggctaagacggctcctggaaagaagaggcctgtagagcagtctcctcaggaaccggactcctccgcgggtattggcaaatcgggtgcacagcccgctaaaaagagactcaatttcggtcagactggcgacacagagtcagtcccagaccctcaaccaatcggagaacctcccgcagccccctcaggtgtgggatctcttacaatggcttcaggtggtggcgcaccagtggcagacaataacgaaggtgccgatggagtgggtagttcctcgggaaattggcattgcgattcccaatggctgggggacagagtcatcaccaccagcacccgaacctgggccctgcccacctacaacaatcacctctacaagcaaatctccaacagcacatctggaggatcttcaaatgacaacgcctacttcggctacagcaccccctgggggtattttgacttcaacagattccactgccacttctcaccacgtgactggcagcgactcatcaacaacaactggggattccggcctaagcgactcaacttcaagctcttcaacattcaggtcaaagaggttacggacaacaatggagtcaagaccatcgccaataaccttaccagcacggtccaggtcttcacggactcagactatcagctcccgtacgtgctcgggtcggctcacgagggctgcctcccgccgttcccagcggacgttttcatgattcctcagtacgggtatctgacgcttaatgatggaagccaggccgtgggtcgttcgtccttttactgcctggaatatttcccgtcgcaaatgctaagaacgggtaacaacttccagttcagctacgagtttgagaacgtacctttccatagcagctacgctcacagccaaagcctggaccgactaatgaatccactcatcgaccaatacttgtactatctctcaaagactattaacggttctggacagaatcaacaaacgctaaaattcagtgtggccggacccagcaacatggctgtccagggaagaaactacatacctggacccagctaccgacaacaacgtgtctcaaccactgtgactcaaaacaacaacagcgaatttgcttggcctggagcttcttcttgggctctcaatggacgtaatagcttgatgaatcctggacctgctatggccagccacaaagaaggagaggaccgtttctttcctttgtctggatctttaatttttggcaaacaaggaactggaagagacaacgtggatgcggacaaagtcatgataaccaacgaagaagaaattaaaactactaacccggtagcaacggagtcctatggacaagtggccacaaaccaccagagtgcccaagcacaggcgcagaccggctgggttcaaaaccaaggaatacttccgggtatggtttggcaggacagagatgtgtacctgcaaggacccatttgggccaaaattcctcacacggacggcaactttcacccttctccgctgatgggagggtttggaatgaagcacccgcctcctcagatcctcatcaaaaacacacctgtacctgcggatcctccaacggccttcaacaaggacaagctgaactctttcatcacccagtattctactggccaagtcagcgtggagatcgagtgggagctgcagaaggaaaacagcaagcgctggaacccggagatccagtacacttccaactattacaagtctaataatgttgaatttgctgttaatactgaaggtgtatatagtgaaccccgccccattggcaccagatacctgactcgtaatctgtaattgcttgttaatcaataaaccgtttaattcgtttcagttgaactttggtctctgcgtatttctttcttatctagtttccatggctacgtagataagtagcatggcgggttaatcattaactacagcccgggcgtttaaacagcgggcggaggggtggagtcgtgacgtgaattacgtcatagggttagggaggtcctgtattagaggtcacgtgagtgttttgcgacattttgcgacaccatgtggtctcgctgggggggggggcccgagtgagcacgcagggtctccattttgaagcgggaggtttgaacgagcgctcggaccgggcgcgctcactggccgtcgttttacaacgtcgtgactgggaaaaccctgtaca

SEQ ID NO: 5 - DNA, 16 bp, Artificial Sequence
  Nucleic acid sequence of forward primer, primer SI-1, synthetic sequence
gccagccatctgttgt

SEQ ID NO: 6 - DNA, 16 bp, Artificial Sequence
  Nucleic acid sequence of reverse primer, primer SI-2, synthetic sequence
ggagtggcaccttcca

SEQ ID NO: 7 - DNA, 21 bp, Artificial Sequence
  Nucleic acid sequence of probe SI-1, synthetic sequence
tcccccgtgccttccttgacc

SEQ ID NO: 8 - DNA, 21 bp, Artificial Sequence
  Nucleic acid sequence of forward primer, primer SI-3, synthetic sequence
ggaacccctagtgatggagtt

SEQ ID NO: 9 - DNA, 16 bp, Artificial Sequence
  Nucleic acid sequence of reverse primer, primer SI-4, synthetic sequence
cggcctcagtgagcga

SEQ ID NO: 10 - DNA, 21 bp, Artificial Sequence
  Nucleic acid sequence of probe SI-2, synthetic sequence
cactccctctctgcgcgctcg